European Patent Application EP 4 674 425 A1, published January 7, 2026. Title: 펩타이드를 포함하는 당뇨망막병증의 치료용 조성물. Applicant: 주식회사 아이바이오코리아. Application KR. The sequence listing filed with the application follows.

SEQUENCE LISTING (1 sequence)

SEQ ID NO: 1 - protein, 21 aa, synthetic construct
HYPGLYGLNGLUAIBLEUALA